European Patent Specification EP 3 250 608 B1, published August 21, 2024. Title: CD1d. Applicant: VUMC. The sequence listing filed with the application follows.

SEQUENCE LISTING (84 sequences)

SEQ ID NO: 1 - protein, 126 aa, Artificial Sequence
  full length
VQLVESGGGLVQAGGSLRLSCAASGSSFSSYTMGWFRQAPGKEREIVAAIRWSGESPYYADSVKGRFTISRDNAKNTLYLQMNSLKPEDTAVYFCAARLVPPGIPIERSLENMNYWGKGTLVTVSS

SEQ ID NO: 2 - protein, 126 aa, Artificial Sequence
  fl
VQLVESGGGSVQAGGSLRLSCAASGRSFSSYTMGWCRQAPGKERECVAVIRWSGESPYYADSVKGRFTISRDNAKNTVYLQMNSLKPEDTAVYYCAARLVPPGIPIERTLESMNYWGKGTLVTVSS

SEQ ID NO: 3 - protein, 127 aa, Artificial Sequence
  fl
QVQLVESGGGLVQAGGSLRLSCAASGSSFSSYTMGWFRQAPGKEREIVAAIRWSGESPIYADSVKGRFTISRDNAKNTLYLQMNSLKPEDTAVYYCAARLVPPGIPIERTLESMRYWGKGTLVTVSS

SEQ ID NO: 4 - protein, 130 aa, Artificial Sequence
  fl
EVQLVESGGGLVQAGGSLGLSCAASGRSFSSYTMGVIRWSGESPYYADSVKGAIRWSGESPYYADSVKGRFTISRDNAKNTLYLQMNNLKPEDTAVYYCAARLVPPGIPIERTLESMKDWGKGTLVTVSS

SEQ ID NO: 5 - protein, 129 aa, Artificial Sequence
  fl
VQLVESGGGLVQAGGSLRLSCAASGSSFSSYTMGAIRWSDESPIYAGSVKGGIRWSDESPIYADSVKGRFTISRDNAKNTLYLQMNSLKPEDTAVYYCAARLVPPGIPIPRTSESMRYWGKGTLVTVSS

SEQ ID NO: 6 - protein, 130 aa, Artificial Sequence
  fl
QVQLVESGGGLVQAGDSLRLSCAASGSSFSSYTMAAIRWSDESPYYSDSVKGAIRWSGESPIYADSVKGRFTISRDNAKNTLYLQMNSLKPEDTAVYNCAARLVPPGIPIERTLESMRYWGKGTLVTVSS

SEQ ID NO: 7 - protein, 129 aa, Artificial Sequence
  fl
EVQLVESGGGLVQAGGSLRLSCAASVSSFSSYTMGTIRTGGSTNYADSVKGGIRWDDENPYYADSVKGRFTISRDNAKNTLYLQMNSLKPEDTANYYCAARLVPPGIPFERTLENMRYWGKGTLVTVSS

SEQ ID NO: 8 - protein, 130 aa, Artificial Sequence
  fl
EVQLVESGGGLVQAGGSLRLSCAASGSSFSSYTMGAIRWSGESPYYADSVKGAIRWDGESPIYAESVKGRFTISRDNAKNTLYLQMNSLKPEDTAVYYCAARLVPPGIPIERTLESMRYWGKGTLVTVSS

SEQ ID NO: 9 - protein, 130 aa, Artificial Sequence
  fl
EVQLVESGGGSVQAGGSLRLSCAASGRSFSSYTMGAIRWSGESPYYADSVKGVIRWSGESPYYADSVKGRFTISRDNAKNTVYLQMASLKPDDTAVYYCAARLVPPGIPIERTLESMNYWGKGTLVTVSS

SEQ ID NO: 10 - protein, 130 aa, Artificial Sequence
  fl
QVQLVESGGGLVQAGGSLRLSCAASGSSFSSYTMGAIRWSGESPYYADSVKGAIRWSDESPIYAGSVKGRFTISRDNAKNTLYLQMNSLKPEDTAVYYCAARLVPPGIPIERTLESMRYWGKGTLVTVSS

SEQ ID NO: 11 - protein, 129 aa, Artificial Sequence
  fl
EVQLVESGGGLVQAGGSLRLSCAASGSSFSSYTMGSINNGGSTKYADSVKGAIRWSDESPYYSDSVKGRFTISRDNAKNTLYLQMNSLKPEDTAVYYCSARLVPPGIPIERTLENMRYSGKGTLVTVSS

SEQ ID NO: 12 - protein, 122 aa, Artificial Sequence
  fl
QVQLVESGGGLVQAGGSLRLSCAASGSMFSDNVMGAIRWSGESPYYVDSVKGTIRTGGSTNYADSVKGRFTISRDNAKNTVYLQMNSLKPEDTAVYYCRHTIPVPSTPYDYWGQGTQVTVSS

SEQ ID NO: 13 - protein, 130 aa, Artificial Sequence
  fl
QVQLVESGGGLVQAGGSLGLSCAASGRSFSSYTMGAIRWSGESPIYADSVKGAIRWSGESPYYADSVKGRFTISRDNAKNTLYLQMNSLKPEDTAVYYCAARLVPPGIPIERTLENMNYWGKGTLVTVSS

SEQ ID NO: 14 - protein, 129 aa, Artificial Sequence
  fl
VQLVESGGGLVQAGGSLRLSCAASGSSFSSYTMGGIRWSGESPYYADSVKGAIRWSGESPYYADSVKGRFTISRDNAKNTLYLQMNSLKPEDTAVYYCAARLVPPGIPIERTLESMNYWGKGTLVTVSS

SEQ ID NO: 15 - protein, 130 aa, Artificial Sequence
  fl
QVQLVESGGGLVQAGGSLRLSCAASGSSFSSYTMGAIRWSGESPYYADSVKGAIRWSGESPIYADSVKGRFTISRDNAKNTLYLQMNSLKPEDTAVYYCAARLVPPGIPIERTLESMKDWGKGTLVTVSS

SEQ ID NO: 16 - protein, 129 aa, Artificial Sequence
  fl
QVQLVESGGGLVQAGGSLRLSCAASGSSFSSYTMTVISSSGSTNYADSVKGGIRWSGESPYYADSVKGRFTISRDNAKNTLYLQMNSLKPEDTAVYYCAARLVPPGIPIERTLESMRYWGKGTLVTVSS

SEQ ID NO: 17 - protein, 129 aa, Artificial Sequence
  fl
VQLVESGGGLVQAGGSLRLSCAASGSSFSSYTMGVIRWSGESPYYADSVKGAIRWSGESPYYGDSVKGRFTISRDNAKNTLYLQMNSLKPEDTAVYYCAARLVPPGIPIGRTLESMNNWGKGTLVTVSS

SEQ ID NO: 18 - protein, 130 aa, Artificial Sequence
  fl
QVQLVESGGGLVQAGGSLRLSCAASGSSFSSYTMGAIRWSDESPIYAGSVKGAIRWSGESPYYADSVKGRFTISRDNAKNTLYLQMHSLKPEDTAVYYCAARLVPPGIPIERALENMNYWGKGTLVTVSS

SEQ ID NO: 19 - protein, 130 aa, Artificial Sequence
  fl
EVQLVESGGGLVQAGGSLRLSCAASGSSFSSYTMGAIRWSDESPYYSDSVKGAIRWSDESPIYADSVKGRFTISRDNAKNTLYLQMHSLKPEDTAFYYCAARLVPPGIPIERTLESMRYWGKGTLVTVSS

SEQ ID NO: 20 - protein, 129 aa, Artificial Sequence
  fl
EVQLVESGGGLVQAGGSLRLSCAASGRSFSSYTMGTIRTGGSTNYADSVKGAIRWSGESPYYADSVKGRFTISRDNAKNTNYLQMNSLKPELTAVYYCAARLVPPGIPIERSLENMNYWGKGTLVTVSS

SEQ ID NO: 21 - protein, 121 aa, Artificial Sequence
  fl
QVQLVESGGGLVQAGGSLRLSCAASGSIFSINAMGAIRWSGESPYYADSVKGVISSSGSTNYADSVKGRFTISRDNAKNTAYLQMNSLKVEDTAVYYCAAHVAGFDEYNYWGQGTQVTVSS

SEQ ID NO: 22 - protein, 10 aa, Artificial Sequence
  1
GSSFSSYTMG

SEQ ID NO: 23 - protein, 10 aa, Artificial Sequence
  1
GRSFSSYTMG

SEQ ID NO: 24 - protein, 10 aa, Artificial Sequence
  1
GSSFSSYTMG

SEQ ID NO: 25 - protein, 10 aa, Artificial Sequence
  1
GRSFSSYTMG

SEQ ID NO: 26 - protein, 10 aa, Artificial Sequence
  1
GSSFSSYTMG

SEQ ID NO: 27 - protein, 10 aa, Artificial Sequence
  1
GSSFSSYTMA

SEQ ID NO: 28 - protein, 10 aa, Artificial Sequence
  1
VSSFSSYTMG

SEQ ID NO: 29 - protein, 10 aa, Artificial Sequence
  1
GSSFSSYTMG

SEQ ID NO: 30 - protein, 10 aa, Artificial Sequence
  1
GRSFSSYTMG

SEQ ID NO: 31 - protein, 10 aa, Artificial Sequence
  1
GSSFSSYTMG

SEQ ID NO: 32 - protein, 10 aa, Artificial Sequence
  1
GSSFSSYTMG

SEQ ID NO: 33 - protein, 10 aa, Artificial Sequence
  1
GSMFSDNVMG

SEQ ID NO: 34 - protein, 10 aa, Artificial Sequence
  1
GRSFSSYTMG

SEQ ID NO: 35 - protein, 10 aa, Artificial Sequence
  1
GSSFSSYTMG

SEQ ID NO: 36 - protein, 10 aa, Artificial Sequence
  1
GSSFSSYTMG

SEQ ID NO: 37 - protein, 10 aa, Artificial Sequence
  1
GSSFSSYTMT

SEQ ID NO: 38 - protein, 10 aa, Artificial Sequence
  1
GSSFSSYTMG

SEQ ID NO: 39 - protein, 10 aa, Artificial Sequence
  1
GSSFSSYTMG

SEQ ID NO: 40 - protein, 10 aa, Artificial Sequence
  1
GSSFSSYTMG

SEQ ID NO: 41 - protein, 10 aa, Artificial Sequence
  1
GRSFSSYTMG

SEQ ID NO: 42 - protein, 10 aa, Artificial Sequence
  1
GSIFSINAMG

SEQ ID NO: 43 - protein, 17 aa, Artificial Sequence
  2
AIRWSGESPYYADSVKG

SEQ ID NO: 44 - protein, 17 aa, Artificial Sequence
  2
VIRWSGESPYYADSVKG

SEQ ID NO: 45 - protein, 17 aa, Artificial Sequence
  2
AIRWSGESPIYADSVKG

SEQ ID NO: 46 - protein, 17 aa, Artificial Sequence
  2
AIRWSGESPYYADSVKG

SEQ ID NO: 47 - protein, 17 aa, Artificial Sequence
  2
GIRWSDESPIYADSVKG

SEQ ID NO: 48 - protein, 17 aa, Artificial Sequence
  2
AIRWSGESPIYADSVKG

SEQ ID NO: 49 - protein, 17 aa, Artificial Sequence
  2
GIRWDDENPYYADSVKG

SEQ ID NO: 50 - protein, 17 aa, Artificial Sequence
  2
AIRWDGESPIYAESVKG

SEQ ID NO: 51 - protein, 17 aa, Artificial Sequence
  2
VIRWSGESPYYADSVKG

SEQ ID NO: 52 - protein, 17 aa, Artificial Sequence
  2
AIRWSDESPIYAGSVKG

SEQ ID NO: 53 - protein, 17 aa, Artificial Sequence
  2
AIRWSDESPYYSDSVKG

SEQ ID NO: 54 - protein, 16 aa, Artificial Sequence
  2
TIRTGGSTNYADSVKG

SEQ ID NO: 55 - protein, 17 aa, Artificial Sequence
  2
AIRWSGESPYYADSVKG

SEQ ID NO: 56 - protein, 17 aa, Artificial Sequence
  2
AIRWSGESPYYADSVKG

SEQ ID NO: 57 - protein, 17 aa, Artificial Sequence
  2
AIRWSGESPIYADSVKG

SEQ ID NO: 58 - protein, 17 aa, Artificial Sequence
  2
GIRWSGESPYYADSVKG

SEQ ID NO: 59 - protein, 17 aa, Artificial Sequence
  2
AIRWSGESPYYGDSVKG

SEQ ID NO: 60 - protein, 17 aa, Artificial Sequence
  2
AIRWSGESPYYADSVKG

SEQ ID NO: 61 - protein, 17 aa, Artificial Sequence
  2
AIRWSDESPIYADSVKG

SEQ ID NO: 62 - protein, 17 aa, Artificial Sequence
  2
AIRWSGESPYYADSVKG

SEQ ID NO: 63 - protein, 16 aa, Artificial Sequence
  2
VISSSGSTNYADSVKG

SEQ ID NO: 64 - protein, 19 aa, Artificial Sequence
  3
RLVPPGIPIERSLENMNYW

SEQ ID NO: 65 - protein, 19 aa, Artificial Sequence
  3
RLVPPGIPIERTLESMNYW

SEQ ID NO: 66 - protein, 19 aa, Artificial Sequence
  3
RLVPPGIPIERTLESMRYW

SEQ ID NO: 67 - protein, 19 aa, Artificial Sequence
  3
RLVPPGIPIERTLESMKDW

SEQ ID NO: 68 - protein, 19 aa, Artificial Sequence
  3
RLVPPGIPIPRTSESMRYW

SEQ ID NO: 69 - protein, 19 aa, Artificial Sequence
  3
RLVPPGIPIERTLESMRYW

SEQ ID NO: 70 - protein, 19 aa, Artificial Sequence
  3
RLVPPGIPFERTLENMRYW

SEQ ID NO: 71 - protein, 19 aa, Artificial Sequence
  3
RLVPPGIPIERTLESMRYW

SEQ ID NO: 72 - protein, 19 aa, Artificial Sequence
  3
RLVPPGIPIERTLESMNYW

SEQ ID NO: 73 - protein, 19 aa, Artificial Sequence
  3
RLVPPGIPIERTLESMRYW

SEQ ID NO: 74 - protein, 19 aa, Artificial Sequence
  3
RLVPPGIPIERTLENMRYS

SEQ ID NO: 75 - protein, 12 aa, Artificial Sequence
  3
TIPVPSTPYDYW

SEQ ID NO: 76 - protein, 19 aa, Artificial Sequence
  3
RLVPPGIPIERTLENMNYW

SEQ ID NO: 77 - protein, 19 aa, Artificial Sequence
  3
RLVPPGIPIERTLESMNYW

SEQ ID NO: 78 - protein, 19 aa, Artificial Sequence
  3
RLVPPGIPIERTLESMKDW

SEQ ID NO: 79 - protein, 19 aa, Artificial Sequence
  3
RLVPPGIPIERTLESMRYW

SEQ ID NO: 80 - protein, 19 aa, Artificial Sequence
  3
RLVPPGIPIGRTLESMNNW

SEQ ID NO: 81 - protein, 19 aa, Artificial Sequence
  3
RLVPPGIPIERALENMNYW

SEQ ID NO: 82 - protein, 19 aa, Artificial Sequence
  3
RLVPPGIPIERTLESMRYW

SEQ ID NO: 83 - protein, 19 aa, Artificial Sequence
  3
RLVPPGIPIERSLENMNYW

SEQ ID NO: 84 - protein, 11 aa, Artificial Sequence
  3
HVAGFDEYNYW